European Patent Application EP 4 545 648 A1, published April 30, 2025. Title: Method for amplifying target nucleic acid using beta-hydroxy acid. Applicant: Seegene, Inc. Application KR. The sequence listing filed with the application follows.

SEQUENCE LISTING (6 sequences)

SEQ ID NO: 1 - DNA, 19 bp, synthetic construct
  source 1..19: mol_type = other DNA
gcgcaacgcaattaatgtg

SEQ ID NO: 2 - DNA, 18 bp, synthetic construct
  source 1..18: mol_type = other DNA
gtaaaacgacggccagtg

SEQ ID NO: 3 - DNA, 41 bp, synthetic construct
  source 1..41: mol_type = other DNA
acaacatacgagccggaagcaagttagctcactcattaggc

SEQ ID NO: 4 - DNA, 42 bp, synthetic construct
  source 1..42: mol_type = other DNA
acacaggaaacagctatgaccacaggtcgactctagaggatc

SEQ ID NO: 5 - DNA, 18 bp, synthetic construct
  source 1..18: mol_type = other DNA
gcgaaagggggatgtgct

SEQ ID NO: 6 - DNA, 18 bp, synthetic construct
  source 1..18: mol_type = other DNA
agttgcgcagcctgaatg